European Patent Specification EP 3 359 558 B1, published December 13, 2023. Title: Borrelia Immunoassays and Materials Therefor. Applicant: BIO-RAD LABORATORIES, INC. The sequence listing filed with the application follows.

SEQUENCE LISTING (12 sequences)

SEQ ID NO: 1 - protein, 6 aa, Artificial Sequence
  Polyhistidine-tag
HHHHHH

SEQ ID NO: 2 - protein, 34 aa, Artificial Sequence
  synthetic fusion peptide
CVQEGVQQEGAQQPGGGMKKNDQIVAAIALRGVA

SEQ ID NO: 3 - protein, 35 aa, Artificial Sequence
  synthetic fusion peptide
KIEFSKFTVKIKNKDGGGMKKNDQIVAAIALRGVA

SEQ ID NO: 4 - protein, 35 aa, Artificial Sequence
  synthetic fusion peptide
DTGSERSIRYRRRVYGGGMKKNDQIVAAIALRGVA

SEQ ID NO: 5 - protein, 193 aa, Borrelia burgdorferi
MTLFLFISCNNSGKDGNTSANSADESVKGPNLTEISKKITDSNAVLLAVKEVEALLSSIDELAKAIGKKIKNDGSLDNEANRNESLLAGAYTISTLITQKLSKLNGSEGLKEKIAAAKKCSEEFSTKLKDNHAQLGIQGVTDENAKKAILKANAAGKDKGVEELEKLSSLESLSKAAKEMLANSVKELTSPVV

SEQ ID NO: 6 - protein, 191 aa, Borrelia burgdorferi
MTLFLFISCNNSGKDGNTSANSADESVKGPNLTEISKKITESNAVVLAVKEVETLLTSIDELAKAIGKKIKNDVSLDNEADHNGSLISGAYLISNLITKKISAIKDSGELKAEIEKAKKCSEEFTAKLKGEHTDLGKEGVTDDNAKKAILKTNNDKTKGADELEKLFESVKNLSKAAKEMLTNSVKELTSP

SEQ ID NO: 7 - protein, 170 aa, Borrelia afzelii
MIKYNKIILTLTLLASLLAACSLTGKARLESSVKDITNEIEKAIKEAEDAGVKTDAFTETQTGGKVAGPKIRAAKIRVADLTIKFLEATEEETITFKENGAGEDEFSGIYDLILNAAKAVEKIGMKDMTKTVEEAAKENPKTTANGIIEIVKVMKAKVENIKEKQTKNQK

SEQ ID NO: 8 - protein, 527 aa, Borrelia garinii
MKLQKLLFSVIFFLTFLCCNKEEKKEGISFKISLGSEPSSLDPQLADDNVGSKMIDTMFRGLITGDPNTGGNKPGLAKSWDISPDGTVYTFTLREKIIWSDGVAITAEGIRKSYLRILNKETGSNYAEMVKSTIKNGQKYFDGQVSDSELGIRAIDEKTLEITLESPKPYFIDMLVHQSFIPIPIHIAEKYGQSWTSPENIVTSGPFKLKERIPNEKYVVEKNDKYYNSNQVEVQEITFYTTNDSSTAYKMYENKELDAIFGSIPPDLIKDLKLRSDYYSSAVNAIYFYAFNTYIKPLDNVKVRKALTLAIDRETLTYKVLDNGTTPTRRIAPNFSSYSYAKNLELFNPEIAKTLLAEAGYPNGNGFPILKLKYNTSEAHKKICEFIQNQWKKILNIDVELENEEWTTYLNTRSNGNYEIARAGWIGDYADPLTFLSIFTQGYTQFSSHNYSSPEYNELIKKSDLELDPIKRQDILRKAEEIIIEKDFPIAPIYIYGNSYLFRNDKWTGWNTNITERFDLSQLKLKN

SEQ ID NO: 9 - protein, 6 aa, Artificial Sequence
  linker
GGSGSG

SEQ ID NO: 10 - protein, 18 aa, Artificial Sequence
  linker
GSTSGSGKPGSGEGSTKG

SEQ ID NO: 11 - protein, 7 aa, Artificial Sequence
  linker
SGRAHAG

SEQ ID NO: 12 - protein, 4 aa, Artificial Sequence
  linker
GSSG